European Patent Application EP 4 242 317 A1, published September 13, 2023. Title: Method for producing reversible immortalized cells. Applicant: National University Corporation Tottori University. The sequence listing filed with the application follows.

SEQUENCE LISTING (4 sequences)

SEQ ID NO: 1 - DNA, 975 bp, Mus musculus
atgcaccggaccacccggatcaagatcaccgagctgaacccccacctgatgtgcgtgctgtgcggcggctacttcatcgacgccaccaccatcatcgagtgcctgcacagcttctgcaagacctgcatcgtgcgctacctggaaaccagcaagtactgccccatctgcgacgtgcaggtgcacaagaccagacccctgctgaacatcagaagcgacaagaccctgcaggacatcgtgtacaagctggtgcccggcctgttcaagaacgagatgaagcggcggagagacttctacgccgcccacccttctgccgatgccgccaatggcagcaacgaggacagaggcgaggtggccgacgaggaaaagcggatcatcaccgacgacgagatcatcagcctgagcatcgagttcttcgaccagagccggctggaccggaaagtgaacaaagagaagcccaaagaagaagtgaacgacaagagatacctgcggtgccctgccgccatgaccgtgatgcacctgagaaagtttctgcggagcaagatggacatccccaacaccttccagatcgacgtgatgtacgaggaagaacccctgaaggactactacaccctgatggatatcgcctacatctacacctggcggcggaacggccctctgcccctgaagtatagagtgcggcctacctgcaagcggatgaagatgagccaccagcgggacggcctgaccaatgccggcgagctggaaagcgatagcggcagcgacaaggccaactctcctgctggcggcgtgccaagcacaagcagctgtctgcctagccccagcacccctgtgcagtctccccaccctcagttcccccacatcagcagcaccatgaacggcaccagcaacagccccagcgccaaccaccagagcagcttcgccagcagacccagaaagagcagcctgaacggcagctccgccaccagctctggatga

SEQ ID NO: 2 - DNA, 3399 bp, Homo sapiens
atgcccagagcccctagatgtagagccgtgcggagcctgctgcggagccactatagagaggtgctgcccctggccaccttcgtgcggagactgggacctcagggatggcggctggtgcagagaggcgatcctgccgcttttagagccctggtggcccagtgtctcgtgtgcgtgccatgggatgccagaccacctcctgccgcccctagcttcagacaggtgtcctgcctgaaagaactggtggccagagtgctgcagcggctgtgtgaaaggggcgccaagaacgtgctggccttcggctttgctctgctggatggcgctagaggcggaccccctgaggcctttacaaccagcgtgcggtcctacctgcccaacaccgtgaccgatgccctgagaggatctggcgcttggggactgctgctgagaagagtgggcgacgacgtgctggtgcatctgctggctagatgcgccctgtttgtgctggtggctcccagctgtgcctaccaagtgtgcggccctccactgtaccagctgggcgctgctacacaggccagacctccacctcatgccagcggccctagaagaaggctgggctgcgagagagcctggaaccactctgtgcgggaagctggggtgccactgggactgcctgcaccaggcgcaagaagaagaggcggcagcgcctctagaagcctgcccctgcccaagaggcctagaagaggggctgctcccgagcccgagagaacacctgtgggacagggatcttgggcccaccccggcagaacaagaggccctagcgatagaggcttctgcgtggtgtcccctgccagacctgccgaggaagccacatctctggaaggcgccctgagcggcacaagacactctcacccaagcgtgggcagacagcaccatgccggcccacctagcacaagcagaccccccagaccttgggacaccccttgccctccagtgtatgccgagacaaagcacttcctgtacagcagcggcgacaaagagcagctgcggcctagcttcctgctgagcagcctgaggccaagcctgaccggcgctagacggctggtggaaaccatcttcctgggcagcagaccctggatgcccggcacacctagaaggctgcctagactgccccagcggtactggcagatgaggcccctgttcctggaactgctgggcaaccatgcccagtgcccttacggcgtgctgctgaaaacccactgccctctgagagccgccgtgacaccagctgctggcgtgtgtgccagagagaagcctcagggctctgtggccgctcccgaggaagaggacaccgatcctcgcagactggtgcagctgctgagacagcacagcagcccttggcaggtgtacggctttgtgcgggcctgcctgagaaggctggtgcctcctggactgtggggcagcaggcacaacgagcggcggtttctgcggaacaccaagaagttcatcagcctgggcaagcacgccaagctgagcctgcaggaactgacctggaagatgagcgtgcggggctgtgcttggctgagaaggtcccctggcgtgggatgtgtgcctgccgccgaacacagactgcgggaagagatcctggccaagtttctgcactggctgatgtccgtgtacgtggtggaactgctgcggagtttcttctacgtgaccgagacaaccttccagaagaaccggctgttcttctaccggaagtccgtgtggtccaagctgcagagcatcggcatccgccagcacctgaagagagtgcagctgagagagctgagcgaggccgaagtgcggcagcacagagaagctagacctgccctgctgaccagcaggctgcggttcatccctaagcccgacggactgcggcccatcgtgaacatggactatgtcgtgggcgccaggaccttcagaagagagaagagagccgagcggctgacctccagagtgaaggccctgttcagcgtgctgaactacgagcgggccagaaggccaggactgctgggagcttctgtgctgggactggacgacatccatagagcctggcggacctttgtgctgagagtgcgggctcaggaccccccacctgagctgtacttcgtgaaggtggacgtgacaggcgcctacgacaccatcccccaggacagactgaccgaagtgatcgccagcatcatcaagccccagaacacctactgtgtgcggagatacgccgtggtgcagaaagccgcccatggccacgtgcgcaaggccttcaagagccacgtgtccaccctgaccgacctgcagccctacatgagacagttcgtggcccatctgcaggaaaccagccccctgagagatgccgtcgtgatcgagcagagcagctccctgaatgaggccagctccggcctgttcgacgtgttcctgagattcatgtgccaccatgctgtgcggatccggggcaagagctacgtgcagtgccagggaatcccacagggcagcatcctgagcaccctgctgtgtagcctgtgctacggcgacatggaaaacaagctgttcgccggcatccggcgggatggcctgctgctgaggctggtggatgacttcctgctcgtgacccctcatctgacccacgccaagacctttctgagaaccctcgtgcggggagtgcccgagtatggctgtgtcgtgaacctgagaaagaccgtcgtgaacttccccgtggaagatgaagccctgggcggcaccgccttcgtgcagatgcctgcccatggactgttcccttggtgcgggctgctgctggacaccagaaccctggaagtgcagagcgactacagcagctacgcccggaccagcatcagagccagcctgaccttcaaccggggcttcaaggccggcagaaacatgcggcggaagctgtttggagtgctgcggctgaagtgccactctctgttcctggatctgcaagtgaacagcctgcagaccgtgtgcaccaacatctacaagatactgctgctgcaggcctaccggttccacgcctgtgtgctgcagctgccattccatcagcaagtgtggaagaaccctacattcttcctgagagtgatcagcgacaccgccagcctgtgttactccatcctgaaggccaaaaacgccggcatgagcctgggagctaaaggcgctgcaggacccctgccttctgaggctgtgcagtggctgtgccatcaggcctttctgctgaagctgaccagacacagagtgacctacgtgcccctgctgggctccctgagaacagcccagacccagctgtccagaaagctgcctggcaccacactgaccgccctggaagccgctgctaatccagccctgcccagcgacttcaagaccatcctggattga

SEQ ID NO: 3 - DNA, 2130 bp, Macaca mulatta polyomavirus
atggataaagttttaaacagagaggaatctttgcagctaatggaccttctaggtcttgaaaggagtgcctgggggaatattcctctgatgagaaaggcatatttaaagaaatgcaaggagtttcatcctgataaaggaggagatgaagaaaagatgaagaaaatgaatactctgtacaagaaaatggaagatggagtaaaatatgctcatcaacctgactttggaggcttctgggatgcaactgagattccaacctatggaactgatgaatgggagcagtggtggaatgcctttaatgaggaaaacctgttttgctcagaagaaatgccatctagtgatgatgaggctactgctgactctcaacattctactcctccaaagaagaagagaaaggtagaagaccccaaggactttccttcagaattgctaagtttcttgagtcatgctgtgtttagtaatagaactcttgcttgctttgctatttacaccacaaaggaaaaagctgcactgctatacaagaaaattatggaaaaatattctgtaacctttataagtaggcataacagttataatcataacatactgttctttcttactccacacaggcatagagtgtctgctattaataactatgctcaaaaattgtgtacctttagctttttaatttgtaaaggggttaataaggaatatttgatgtatagtgccttgactagagatccattttctgttattgaggaaagtttgccaggtgggttaaaggagcatgattttaatccagaagaagcagaggaaactaaacaagtgtcctggaagcttgtaacagagtatgcaatggaaacaaaatgtgatgatgtgttgttattgcttgggatgtacttggaatttcaatacagttttgaaatgtgtttaaaatgtattaagaaagaacagcccagccactataagtaccatgaaaagcattatgcaaatgctgctatatttgctgacagcaaaaaccagaaaaccatatgccaacaggctgttgatactgttttagctaaaaagcgggttgatagcctacaactaactagagaacaaatgttaacaaacagatttaatgatcttttggataggatggatataatgtttggttctacaggctctgctgacatagaagaatggatggctggagttgcttggctacactgtttgttgcccaaaatggattcagtggtgtatgactttttaaaatgcatggtgtacaacattcctaagaaaagatactggctgtttaaaggaccaattgatagtggtaaaactacattagcagctgctttgcttgaattatgtggggggaaagctttaaatgttaatttgcccttggacaggctgaactttgagctaggagtagctattgaccagtttttagtagtttttgaggatgtaaagggcactggaggggagtccagagatttgccttcaggtcagggaattaataacctggacaatttaagggattatttggatggcagtgttaaggtaaacttagaaaagaaacacctaaataaaagaactcaaatatttccccctggaatagtcaccatgaatgagtacagtgtgcctaaaacactgcaggccagatttgtaaaacaaatagattttaggcccaaagattatttaaagcattgcctggaacgcagtgagtttttgttagaaaagaggataattcaaagtggcattgctttgcttcttatgttaatttggtacagacctgtggctgagtttgctcaaagtattcagagcagaattgtggagtggaaagagagattggacaaagagtttagtttgtcagtgtatcaaaagatgaagtttaatgtggctatgggaactggagttttagattggctaagaaacagtgataatgatgatgaagacagccaggaaaatgctgataaaaatgaagatggtggggagaagaacatggaagactcagggcatgaaacaggcattgattcacagtctcaaggctcatttcaggcccctcagccctcacagtcctcacagtctgttcatgatcagccatatcacatttgtagaggttttacttgctttaagaaacctcccacacctccccctgaacctgaaacataa

SEQ ID NO: 4 - DNA, 851 bp, Human papillomavirus
gaattcatgcaccaaaagagaactgcaatgtttcaggacccacaggagcgacccagaaagttaccacagttatgcacagagctgcaaacaactatacatgatataatattagaatgtgtgtactgcaagcaacagttactgcgacgtgaggtatatgactttgcttttcgggatttatgcatagtatatagagatgggaatccatatgctgtatgtgataaatgtttaaagttttattctaaaattagtgagtatagacattattgttatagtttgtatggaacaacattagaacagcaatacaacaaaccgttgtgtgatttgttaattaggtgtattaactgtcaaaagccactgtgtcctgaagaaaagcaaagacatctggacaaaaagcaaagattccataatataaggggtcggtggaccggtcgatgtatgtcttgttgcagatcatcaagaacacgtagagaaacccagctgggaagcggagctactaacttcagcctgctgaagcaggctggagacgtggaggagaaccctggacctatgcatggagatacacctacattgcatgaatatatgttagatttgcaaccagagacaactgatctctactgttatgagcaattaaatgacagctcagaggaggaggatgaaatagatggtccagctggacaagcagaaccggacagagcccattacaatattgtaaccttttgttgcaagtgtgactctacgcttcggttgtgcgtacaaagcacacacgtagacattcgtactttggaagacctgttaatgggcacactaggaattgtgtgccccatctgttctcagaaaccataagaattctt